European Patent Specification EP 3 860 630 B1, published January 3, 2024. Title: MICROBIALS FOR ANIMALS. Applicant: MICROBIAL DISCOVERY GROUP, LLC UNITED ANIMAL HEALTH, INC. Application PCT/US2019/054190. The sequence listing filed with the application follows.

SEQUENCE LISTING (3 sequences)

SEQ ID NO: 1 - DNA, 10 bp, Artificial Sequence
  Description of Artificial Sequence: Synthetic primer
ggtgcgggaa

SEQ ID NO: 2 - DNA, 10 bp, Artificial Sequence
  Description of Artificial Sequence: Synthetic primer
gtttcgctcc

SEQ ID NO: 3 - DNA, 10 bp, Artificial Sequence
  Description of Artificial Sequence: Synthetic primer
gtagacccgt